European Patent Application EP 4 154 903 A1, published March 29, 2023. Title: LIVER-SPECIFIC NUCLEIC ACID REGULATORY ELEMENTS AND METHODS AND USE THEREOF. Applicant: VIB VZW. The sequence listing filed with the application follows.

SEQUENCE LISTING (40 sequences)

SEQ ID NO: 1 - DNA, 88 bp, Homo sapiens
  source 1..88: mol_type = unassigned DNA
ggagttgctggtgcttccccaggctggagattgagttaatattaacaggcccaaggcgatgtgggcttgtgcaatcataggcccggcc

SEQ ID NO: 2 - DNA, 41 bp, Homo sapiens
  source 1..41: mol_type = unassigned DNA
atcgccaggtcacctgaggagttaatgaatacatatctcct

SEQ ID NO: 3 - DNA, 72 bp, Homo sapiens
  source 1..72: mol_type = unassigned DNA
gggggaggctgctggtgaatattaaccaaggtcaccccagttatcggaggagcaaacaggggctaagtccac

SEQ ID NO: 4 - DNA, 71 bp, Homo sapiens
  source 1..71: mol_type = unassigned DNA
tgaatgaccttcagcctgttcccgtccctgatatgggcaaacattgcaagcagcaaacagcaaacacatag

SEQ ID NO: 5 - DNA, 173 bp, Homo sapiens
  source 1..173: mol_type = unassigned DNA
ggcgtattcttaagaatagattaaataatcataaaaagatctatacttaaaaattgaaaaatgcttaaatattaaaattcttctcataaaaaaatactaatttaaaaatgagcctgaaatgtttatctatttattgcacagggttgcatacataaaacgacacaccctcttgt

SEQ ID NO: 6 - DNA, 551 bp, Homo sapiens
  source 1..551: mol_type = unassigned DNA
agtttggaacaagactatataccatatcctacaggaagaataaaagtaaaggaaaggtgccatctctactgaatagagagtcctaacaaaaaggcttcaaaaggactctgcatctttaataatataaaaaggctaggacacaaacagcatcatctaaaatgccattagaaatacttcacatacaaaaaggtctaagtaaagcaggattttataaagtgatcaaaaaagaaacactaagggggaaaaatcttttaagattaaagaggtttttcaaaggacaagttgaagtggctgtaaaatttatgaggcagcattaaacttcagttctaagtaacaataaattattcaccataaaaacatacatgtgtcaaatattataagcctcttaaactttttaaaacaatttcttgcagaactgattagatatattaagtcaagattagcagatactaactttttcattagcatactatgatcactcagagtaaaggaggaaatttagaaaagaaataagacagaaccatcaatagtcgattcaccaccaaatgtga

SEQ ID NO: 7 - DNA, 94 bp, Homo sapiens
  source 1..94: mol_type = unassigned DNA
ctaaaatgggcaaacattgcaagcagcaaacagcaaacacacagccctccctgcctgctgaccttggagctggggcagaggtcagagacctctc

SEQ ID NO: 8 - DNA, 101 bp, Homo sapiens
  source 1..101: mol_type = unassigned DNA
cagccaatgaaatacaaagatgagtctagttaataatctacaattattggttaaagaagtatattagtgctaatttccctccgtttgtcctagcttttctc

SEQ ID NO: 9 - DNA, 135 bp, Homo sapiens
  source 1..135: mol_type = unassigned DNA
gcatgattttaaggactggttgtttatgagccaatcagaggtgttgaataaacacctccctactaggtcaaggtagaaaggggagggcaaatattggaaaaaaaaaacatgatgagaagtctataaaaattgtgt

SEQ ID NO: 10 - DNA, 141 bp, Homo sapiens
  source 1..141: mol_type = unassigned DNA
tgcgggaatcagcctttgaaacgatggccaacagcagctaataataaaccagtaatttgggatagacgagtagcaagagggcattggttggtgggtcaccctccttctcagaacacattataaaaaccttccgtttccaca

SEQ ID NO: 11 - DNA, 74 bp, Homo sapiens
  source 1..74: mol_type = unassigned DNA
tgccactcctagttcccatcctatttaaatctgcaagaggtttggttaatcattggctttgtcctgtgtagaca

SEQ ID NO: 12 - DNA, 441 bp, Homo sapiens
  source 1..441: mol_type = unassigned DNA
ttccttcccccttccaagacccccctgaatcctatcaaaagcacatcttccattcattgcttcccggtgtcattatgacaagcggctacaaatcaatagcagagggaaaggcaggaccaacccgcactcaccaagtgataaagattcactctcagccccgatttgctaatagcccataatagcagccattggcgccccgcattaaataatacatttcactccgcgtttattatgggatttttaaaactcctcaccaaattggattttctcgatggtctctaatttccacatttatcatttaaaattaaactgctctgtggaaaggggggatagagaagaagaaggtagagagaggccagacagtactgtatttttccttttgactcccccctttatgaaaacccataaataatatcaggtatcacagctataagcagcagg

SEQ ID NO: 13 - DNA, 171 bp, Homo sapiens
  source 1..171: mol_type = unassigned DNA
aggaggaactgctcaaaacagacagaggctctttgtttgctttgcttctgtgtcaactgggcaacatttggaaacaacaaatattggttcagaggcccactgctttcttacccacctcctgctggtcagcttttccagctttcctgcacgtacacacaagcgcagctattt

SEQ ID NO: 14 - DNA, 170 bp, Homo sapiens
  source 1..170: mol_type = unassigned DNA
cgatgctctaatctctctagacaaggttcatatttgtatgggttacttattctctctttgttgactaagtcaataatcagaatcagcaggtttgcagtcagattggcagggataagcagcctagctcaggagaagtgagtataaaagccccaggctgggagcagccatca

SEQ ID NO: 15 - DNA, 48 bp, synthetic construct
  source 1..48: mol_type = other DNA; note = Forward primer
aagcggccgcggtaccgtctgtctgcacatttcgtagagcgagtgttc

SEQ ID NO: 16 - DNA, 36 bp, synthetic construct
  source 1..36: mol_type = other DNA; note = Reverse primer
agcgctagccaggagcttgtggatctgtgtgacggc

SEQ ID NO: 17 - DNA, 223 bp, synthetic construct
  source 1..223: mol_type = other DNA; note = TTRmin sequence
gtctgtctgcacatttcgtagagcgagtgttccgatactctaatctccctaggcaaggttcatatttgtgtaggttacttattctccttttgttgactaagtcaataatcagaatcagcaggtttggagtcagcttggcagggatcagcagcctgggttggaaggagggggtataaaagccccttcaccaggagaagccgtcacacagatccacaagctcctg

SEQ ID NO: 18 - DNA, 114 bp, synthetic construct
  source 1..114: mol_type = other DNA; note = SEQ ID NO: 1 with restriction site
ggtaccggcgcgccggagttgctggtgcttccccaggctggagattgagttaatattaacaggcccaaggcgatgtgggcttgtgcaatcataggcccggccacgcgtggtacc

SEQ ID NO: 19 - DNA, 67 bp, synthetic construct
  source 1..67: mol_type = other DNA; note = SEQ ID NO: 2 with restriction site
ggtaccggcgcgccatcgccaggtcacctgaggagttaatgaatacatatctcctacgcgtggtacc

SEQ ID NO: 20 - DNA, 98 bp, synthetic construct
  source 1..98: mol_type = other DNA; note = SEQ ID NO: 3 with restriction site
ggtaccggcgcgccgggggaggctgctggtgaatattaaccaaggtcaccccagttatcggaggagcaaacaggggctaagtccacacgcgtggtacc

SEQ ID NO: 21 - DNA, 97 bp, synthetic construct
  source 1..97: mol_type = other DNA; note = SEQ ID NO: 4 with restriction site
ggtaccggcgcgcctgaatgaccttcagcctgttcccgtccctgatatgggcaaacattgcaagcagcaaacagcaaacacatagacgcgtggtacc

SEQ ID NO: 22 - DNA, 199 bp, synthetic construct
  source 1..199: mol_type = other DNA; note = SEQ ID NO: 5 with restriction site
ggtaccggcgcgccggcgtattcttaagaatagattaaataatcataaaaagatctatacttaaaaattgaaaaatgcttaaatattaaaattcttctcataaaaaaatactaatttaaaaatgagcctgaaatgtttatctatttattgcacagggttgcatacataaaacgacacaccctcttgtacgcgtggtacc

SEQ ID NO: 23 - DNA, 576 bp, synthetic construct
  source 1..576: mol_type = other DNA; note = SEQ ID NO: 6 with restriction site
ggtaccggcgcgccagtttggaacaagactatataccatatcctacaggaagaataaaagtaaaggaaaggtgccatctctactgaatagagagtcctaacaaaaaggcttcaaaaggactctgcatctttaataatataaaaaggctaggacacaaacagcatcatctaaaatgccattagaaatacttcacatacaaaaaggtctaagtaaagcaggattttataaagtgatcaaaaaagaaacactaagggggaaaaatcttttaagattaaagaggtttttcaaaggacaagttgaagtggctgtaaaatttatgaggcagcattaaacttcagttctaagtaacaataaattattcaccataaaaacatacatgtgtcaaatattataagcctcttaaactttttaaaacaatttcttgcagaactgattagatatattaagtcaagattagcagatactaactttttcattagcatactatgatcactcagagtaaaggaggaaatttagaaaagaaataagacagaaccatcaatagtcgattcaccaccaaatgtgacgcgtggtacc

SEQ ID NO: 24 - DNA, 119 bp, synthetic construct
  source 1..119: mol_type = other DNA; note = SEQ ID NO: 7 with restriction site
ggtaccggcgcgcctaaaatgggcaaacattgcaagcagcaaacagcaaacacacagccctccctgcctgctgaccttggagctggggcagaggtcagagacctctcacgcgtggtacc

SEQ ID NO: 25 - DNA, 126 bp, synthetic construct
  source 1..126: mol_type = other DNA; note = SEQ ID NO: 8 with restriction site
ggtaccggcgcgccagccaatgaaatacaaagatgagtctagttaataatctacaattattggttaaagaagtatattagtgctaatttccctccgtttgtcctagcttttctcacgcgtggtacc

SEQ ID NO: 26 - DNA, 161 bp, synthetic construct
  source 1..161: mol_type = other DNA; note = SEQ ID NO: 9 with restriction site
ggtaccggcgcgccgcatgattttaaggactggttgtttatgagccaatcagaggtgttgaataaacacctccctactaggtcaaggtagaaaggggagggcaaatattggaaaaaaaaaacatgatgagaagtctataaaaattgtgtacgcgtggtacc

SEQ ID NO: 27 - DNA, 166 bp, synthetic construct
  source 1..166: mol_type = other DNA; note = SEQ ID NO: 10 with restriction site
ggtaccggcgcgcctgcgggaatcagcctttgaaacgatggccaacagcagctaataataaaccagtaatttgggatagacgagtagcaagagggcattggttggtgggtcaccctccttctcagaacacattataaaaaccttccgtttccacacgcgtggtacc

SEQ ID NO: 28 - DNA, 99 bp, synthetic construct
  source 1..99: mol_type = other DNA; note = SEQ ID NO: 11 with restriction site
ggtaccggcgcgcctgccactcctagttcccatcctatttaaatctgcaagaggtttggttaatcattggctttgtcctgtgtagacacgcgtggtacc

SEQ ID NO: 29 - DNA, 467 bp, synthetic construct
  source 1..467: mol_type = other DNA; note = SEQ ID NO: 12 with restriction site
ggtaccggcgcgccttccttcccccttccaagacccccctgaatcctatcaaaagcacatcttccattcattgcttcccggtgtcattatgacaagcggctacaaatcaatagcagagggaaaggcaggaccaacccgcactcaccaagtgataaagattcactctcagccccgatttgctaatagcccataatagcagccattggcgccccgcattaaataatacatttcactccgcgtttattatgggatttttaaaactcctcaccaaattggattttctcgatggtctctaatttccacatttatcatttaaaattaaactgctctgtggaaaggggggatagagaagaagaaggtagagagaggccagacagtactgtatttttccttttgactcccccctttatgaaaacccataaataatatcaggtatcacagctataagcagcaggacgcgtggtacc

SEQ ID NO: 30 - DNA, 197 bp, synthetic construct
  source 1..197: mol_type = other DNA; note = SEQ ID NO: 13 with restriction site
ggtaccggcgcgccaggaggaactgctcaaaacagacagaggctctttgtttgctttgcttctgtgtcaactgggcaacatttggaaacaacaaatattggttcagaggcccactgctttcttacccacctcctgctggtcagcttttccagctttcctgcacgtacacacaagcgcagctatttacgcgtggtacc

SEQ ID NO: 31 - DNA, 194 bp, synthetic construct
  source 1..194: mol_type = other DNA; note = SEQ ID NO: 14 with restriction site
ggtaccggcgcgccgatgctctaatctctctagacaaggttcatatttgtatgggttacttattctctctttgttgactaagtcaataatcagaatcagcaggtttgcagtcagattggcagggataagcagcctagctcaggagaagtgagtataaaagccccaggctgggagcagccatcacgcgtggtacc

SEQ ID NO: 32 - DNA, 22 bp, synthetic construct
  source 1..22: mol_type = other DNA; note = Forward primer
agggatatcgacttgcagaaaa

SEQ ID NO: 33 - DNA, 27 bp, synthetic construct
  source 1..27: mol_type = other DNA; note = Probe
agtcctgtgaaccagcagtgccatttc

SEQ ID NO: 34 - DNA, 25 bp, synthetic construct
  source 1..25: mol_type = other DNA; note = Reverse primer
gtgagcttagaagtttgtgaaacag

SEQ ID NO: 35 - DNA, 20 bp, synthetic construct
  source 1..20: mol_type = other DNA; note = Forward primer
gccttctagttgccagccat

SEQ ID NO: 36 - DNA, 20 bp, synthetic construct
  source 1..20: mol_type = other DNA; note = Probe
tgtttgcccctcccccgtgc

SEQ ID NO: 37 - DNA, 19 bp, synthetic construct
  source 1..19: mol_type = other DNA; note = Reverse primer
ggcaccttccagggtcaag

SEQ ID NO: 38 - DNA, 20 bp, synthetic construct
  source 1..20: mol_type = other DNA; note = Forward primer
tgtgtccgtcgtggatctga

SEQ ID NO: 39 - DNA, 29 bp, synthetic construct
  source 1..29: mol_type = other DNA; note = Probe
cctggagaaacctgccaagtatgatgaca

SEQ ID NO: 40 - DNA, 21 bp, synthetic construct
  source 1..21: mol_type = other DNA; note = Reverse primer
cctgcttcaccaccttcttga